European Patent Application EP 4 678 186 A1, published January 14, 2026. Title: 包含抗CTLA4-抗PD-1双特异性抗体的药物组合及其用途. Applicant: 康方药业有限公司. The sequence listing filed with the application follows.

SEQUENCE LISTING (45 sequences)

SEQ ID NO: 1 - DNA, 372 bp, synthetic construct
  source 1..372: mol_type = other DNA
caggtcaagctgcaggagtctggacctgagctggtgaagcctggagcttcaatgaagatatcctgcaaggcttctggttactcattcactggctacaccatgaactgggtgaagcagagccatggaaagaaccttgaatggattggacttattaatccttacaataatattactaactacaaccagaagttcatgggcaaggccacatttactgtagacaagtcatccagcacagcctacatggaactcctcagactgacatctgaagactctggagtctatttctgtgcaagactcgactataggtcttattggggccaagggactctggtcactgtctctgcagccaaaacgacacccccatctgtctat

SEQ ID NO: 2 - protein, 124 aa, synthetic construct
QVKLQESGPELVKPGASMKISCKASGYSFTGYTMNWVKQSHGKNLEWIGLINPYNNITNYNQKFMGKATFTVDKSSSTAYMELLRLTSEDSGVYFCARLDYRSYWGQGTLVTVSAAKTTPPSVY

SEQ ID NO: 3 - DNA, 378 bp, synthetic construct
  source 1..378: mol_type = other DNA
caggctgttgtgactcaggaatctgcactcaccacatcacctggtgaaacagtcacactcacttgtcgctcaagtactggggctgttacaactagtaactttgccaactgggtccaagaaaaaccagatcatttattcactagtctaataggtggtaccaacaaccgagctccaggtgttcctgccagattctcaggctccctgattggagacaaggctgccctcaccatcacaggggcacagactgaggatgaggcaatatatttctgtgctctatggtacagcaaccattgggtgttcggtggaggaaccaaactgactgtcctaggccagcccaagtcttcgccatcagtcaccctgtttcaagggcaattctgc

SEQ ID NO: 4 - protein, 126 aa, synthetic construct
QAVVTQESALTTSPGETVTLTCRSSTGAVTTSNFANWVQEKPDHLFTSLIGGTNNRAPGVPARFSGSLIGDKAALTITGAQTEDEAIYFCALWYSNHWVFGGGTKLTVLGQPKSSPSVTLFQGQFC

SEQ ID NO: 5 - DNA, 345 bp, synthetic construct
  source 1..345: mol_type = other DNA
caggtgcagctggtggagtctggggccgagctggtgaagcccggcgcctccatgaagatctcttgcaaggccagcggatacagtttcactggctataccatgaactgggtcaaacaggctccaggacagggactggagtggatcgggctgattaatccttacaacaacatcaccaactacaaccagaagttcatgggaaaagcaacctttacagtggacaagagcatttccacagcctacatggaactgagccggctgacttcagacgatagcggggtctatttttgtgcaaggctggattatcgctcttactgggggcagggaactctggtcactgtctccgct

SEQ ID NO: 6 - protein, 115 aa, synthetic construct
QVQLVESGAELVKPGASMKISCKASGYSFTGYTMNWVKQAPGQGLEWIGLINPYNNITNYNQKFMGKATFTVDKSISTAYMELSRLTSDDSGVYFCARLDYRSYWGQGTLVTVSA

SEQ ID NO: 7 - DNA, 327 bp, synthetic construct
  source 1..327: mol_type = other DNA
caggctgtcgtcactcaggaaccttcactgactgtgagcccaggaggaactgtcaccctgacatgcggaagctccaccggagcagtgaccacatccaacttcgccaattgggtccaggaaaagccaggccaggcatttcgatccctgatcggaggcacaaacaatcgggcttcttgggtgcccgcaagattctcaggaagcctgctggggggaaaagccgctctgaccattagtggcgctcagcctgaggacgaagccgagtacttctgcgctctgtggtatagcaaccactgggtgtttggcgggggaacaaagctgactgtgctg

SEQ ID NO: 8 - protein, 109 aa, synthetic construct
QAVVTQEPSLTVSPGGTVTLTCGSSTGAVTTSNFANWVQEKPGQAFRSLIGGTNNRASWVPARFSGSLLGGKAALTISGAQPEDEAEYFCALWYSNHWVFGGGTKLTVL

SEQ ID NO: 9 - DNA, 345 bp, synthetic construct
  source 1..345: mol_type = other DNA
caggtgcagctggtcgagtctggggccgaagtgaagaaacccggcgcctcagtgaaggtcagctgcaaggccagcgggtacagtttcactggatataccatgaactgggtccgacaggcccctggccaggggctggagtggatcggcctgattaacccttacaacaacatcactaactacgcacagaagttccaggggagagtgacctttacagtggacaccagcatttccacagcctacatggaactgtcccggctgagatctgacgatacaggcgtgtacttctgcgctaggctggattaccgcagctattggggacagggcacactggtgactgtcagcgca

SEQ ID NO: 10 - protein, 115 aa, synthetic construct
QVQLVESGAEVKKPGASVKVSCKASGYSFTGYTMNWVRQAPGQGLEWIGLINPYNNITNYAQKFQGRVTFTVDTSISTAYMELSRLRSDDTGVYFCARLDYRSYWGQGTLVTVSA

SEQ ID NO: 11 - DNA, 327 bp, synthetic construct
  source 1..327: mol_type = other DNA
caggctgtcgtcactcaggaaccttcactgaccgtgtctcctggcgggactgtcaccctgacatgcggcagctccacaggggccgtgaccacaagtaacttcccaaattgggtccagcagaagccaggacaggctccccggagtctgatcggaggcaccaacaacaaggccagctggacacccgcacggttcagcggcagcctgctgggcggcaaggccgctctgacaattagcggagcccagcctgaggacgaagccgagtactattgcgctctgtggtactccaaccactgggtgttcggcggcggcaccaagctgactgtgctg

SEQ ID NO: 12 - protein, 109 aa, synthetic construct
QAVVTQEPSLTVSPGGTVTLTCGSSTGAVTTSNFPNWVQQKPGQAPRSLIGGTNNKASWTPARFSGSLLGGKAALTISGAQPEDEAEYYCALWYSNHWVFGGGTKLTVL

SEQ ID NO: 13 - DNA, 354 bp, synthetic construct
  source 1..354: mol_type = other DNA
gaggtcaaactggtggagagcggcggcgggctggtgaagcccggcgggtcactgaaactgagctgcgccgcttccggcttcgcctttagctcctacgacatgtcatgggtgaggcagacccctgagaagcgcctggaatgggtcgctactatcagcggaggcgggcgatacacctactatcctgactctgtcaaagggagattcacaattagtcgggataacgccagaaatactctgtatctgcagatgtctagtctgcggtccgaggatacagctctgtactattgtgcaaaccggtacggcgaagcatggtttgcctattggggacagggcaccctggtgacagtctctgcc

SEQ ID NO: 14 - protein, 118 aa, synthetic construct
EVKLVESGGGLVKPGGSLKLSCAASGFAFSSYDMSWVRQTPEKRLEWVATISGGGRYTYYPDSVKGRFTISRDNARNTLYLQMSSLRSEDTALYYCANRYGEAWFAYWGQGTLVTVSA

SEQ ID NO: 15 - DNA, 321 bp, synthetic construct
  source 1..321: mol_type = other DNA
gacattaagatgacacagtccccttcctcaatgtacgctagcctgggcgagcgagtgaccttcacatgcaaagcatcccaggacatcaacacatacctgtcttggtttcagcagaagccaggcaaaagccccaagaccctgatctaccgggccaatagactggtggacggggtccccagcagattctccggatctggcagtgggcaggattactccctgaccatcagctccctggagtatgaagacatgggcatctactattgcctgcagtatgatgagttccctctgacctttggagcaggcacaaaactggaactgaag

SEQ ID NO: 16 - protein, 107 aa, synthetic construct
DIKMTQSPSSMYASLGERVTFTCKASQDINTYLSWFQQKPGKSPKTLIYRANRLVDGVPSRFSGSGSGQDYSLTISSLEYEDMGIYYCLQYDEFPLTFGAGTKLELK

SEQ ID NO: 17 - DNA, 354 bp, synthetic construct
  source 1..354: mol_type = other DNA
gaagtgcagctggtcgagtctgggggagggctggtgcagcccggcgggtcactgcgactgagctgcgcagcttccggattcgcctttagctcctacgacatgtcctgggtgcgacaggcaccaggaaagggactggattgggtcgctactatctcaggaggcgggagatacacctactatcctgacagcgtcaagggccggttcacaatctctagagataacagtaagaacaatctgtatctgcagatgaacagcctgagggctgaggacaccgcactgtactattgtgccaaccgctacggggaagcatggtttgcctattgggggcagggaaccctggtgacagtctctagt

SEQ ID NO: 18 - protein, 118 aa, synthetic construct
EVQLVESGGGLVQPGGSLRLSCAASGFAFSSYDMSWVRQAPGKGLDWVATISGGGRYTYYPDSVKGRFTISRDNSKNNLYLQMNSLRAEDTALYYCANRYGEAWFAYWGQGTLVTVSS

SEQ ID NO: 19 - DNA, 321 bp, synthetic construct
  source 1..321: mol_type = other DNA
gacattcagatgactcagagcccctcctccatgtccgcctctgtgggcgacagggtcaccttcacatgccgcgctagtcaggatatcaacacctacctgagctggtttcagcagaagccagggaaaagccccaagacactgatctaccgggctaatagactggtgtctggagtcccaagtcggttcagtggctcagggagcggacaggactacactctgaccatcagctccctgcagcctgaggacatggcaacctactattgcctgcagtatgatgagttcccactgacctttggcgccgggacaaaactggagctgaag

SEQ ID NO: 20 - protein, 107 aa, synthetic construct
DIQMTQSPSSMSASVGDRVTFTCRASQDINTYLSWFQQKPGKSPKTLIYRANRLVSGVPSRFSGSGSGQDYTLTISSLQPEDMATYYCLQYDEFPLTFGAGTKLELK

SEQ ID NO: 21 - DNA, 1344 bp, synthetic construct
  source 1..1344: mol_type = other DNA
gaagtgcagctggtcgagtctgggggagggctggtgcagcccggcgggtcactgcgactgagctgcgcagcttccggattcgcctttagctcctacgacatgtcctgggtgcgacaggcaccaggaaagggactggattgggtcgctactatctcaggaggcgggagatacacctactatcctgacagcgtcaagggccggttcacaatctctagagataacagtaagaacaatctgtatctgcagatgaacagcctgagggctgaggacaccgcactgtactattgtgccaaccgctacggggaagcatggtttgcctattgggggcagggaaccctggtgacagtctctagtgccagcaccaaaggacctagcgtgtttcctctcgccccctcctccaaaagcaccagcggaggaaccgctgctctcggatgtctggtgaaggactacttccctgaacccgtcaccgtgagctggaatagcggcgctctgacaagcggagtccatacattccctgctgtgctgcaaagcagcggactctattccctgtccagcgtcgtcacagtgcccagcagcagcctgggcacccagacctacatctgtaacgtcaaccacaagccctccaacaccaaggtggacaagaaagtggagcccaaatcctgcgacaagacacacacctgtcccccctgtcctgctcccgaactcctcggaggccctagcgtcttcctctttcctcccaaacccaaggacaccctcatgatcagcagaacccctgaagtcacctgtgtcgtcgtggatgtcagccatgaggaccccgaggtgaaattcaactggtatgtcgatggcgtcgaggtgcacaacgccaaaaccaagcccagggaggaacagtacaactccacctacagggtggtgtccgtgctgacagtcctccaccaggactggctgaacggcaaggagtacaagtgcaaggtgtccaacaaggctctccctgcccccattgagaagaccatcagcaaggccaaaggccaacccagggagccccaggtctatacactgcctccctccagggacgaactcaccaagaaccaggtgtccctgacctgcctggtcaagggcttttatcccagcgacatcgccgtcgagtgggagtccaacggacagcccgagaataactacaagaccacccctcctgtcctcgactccgacggctccttcttcctgtacagcaagctgaccgtggacaaaagcaggtggcagcagggaaacgtgttctcctgcagcgtgatgcacgaagccctccacaaccactacacccagaaaagcctgtccctgagccccggcaaa

SEQ ID NO: 22 - protein, 448 aa, synthetic construct
EVQLVESGGGLVQPGGSLRLSCAASGFAFSSYDMSWVRQAPGKGLDWVATISGGGRYTYYPDSVKGRFTISRDNSKNNLYLQMNSLRAEDTALYYCANRYGEAWFAYWGQGTLVTVSSASTKGPSVFPLAPSSKSTSGGTAALGCLVKDYFPEPVTVSWNSGALTSGVHTFPAVLQSSGLYSLSSVVTVPSSSLGTQTYICNVNHKPSNTKVDKKVEPKSCDKTHTCPPCPAPELLGGPSVFLFPPKPKDTLMISRTPEVTCVVVDVSHEDPEVKFNWYVDGVEVHNAKTKPREEQYNSTYRVVSVLTVLHQDWLNGKEYKCKVSNKALPAPIEKTISKAKGQPREPQVYTLPPSRDELTKNQVSLTCLVKGFYPSDIAVEWESNGQPENNYKTTPPVLDSDGSFFLYSKLTVDKSRWQQGNVFSCSVMHEALHNHYTQKSLSLSPGK

SEQ ID NO: 23 - DNA, 642 bp, synthetic construct
  source 1..642: mol_type = other DNA
gacattcagatgactcagagcccctcctccatgtccgcctctgtgggcgacagggtcaccttcacatgccgcgctagtcaggatatcaacacctacctgagctggtttcagcagaagccagggaaaagccccaagacactgatctaccgggctaatagactggtgtctggagtcccaagtcggttcagtggctcagggagcggacaggactacactctgaccatcagctccctgcagcctgaggacatggcaacctactattgcctgcagtatgatgagttcccactgacctttggcgccgggacaaaactggagctgaagcgaactgtggccgctccctccgtcttcatttttcccccttctgacgaacagctgaaatcaggcacagccagcgtggtctgtctgctgaacaatttctaccctagagaggcaaaagtgcagtggaaggtcgataacgccctgcagtccggcaacagccaggagagtgtgactgaacaggactcaaaagatagcacctattccctgtctagtacactgactctgtccaaggctgattacgagaagcacaaagtgtatgcatgcgaagtgacacatcagggactgtcaagccccgtgactaagtcttttaaccggggcgaatgt

SEQ ID NO: 24 - protein, 214 aa, synthetic construct
DIQMTQSPSSMSASVGDRVTFTCRASQDINTYLSWFQQKPGKSPKTLIYRANRLVSGVPSRFSGSGSGQDYTLTISSLQPEDMATYYCLQYDEFPLTFGAGTKLELKRTVAAPSVFIFPPSDEQLKSGTASVVCLLNNFYPREAKVQWKVDNALQSGNSQESVTEQDSKDSTYSLSSTLTLSKADYEKHKVYACEVTHQGLSSPVTKSFNRGEC

SEQ ID NO: 25 - protein, 15 aa, synthetic construct
GGGGSGGGGSGGGGS

SEQ ID NO: 26 - protein, 20 aa, synthetic construct
GGGGSGGGGSGGGGSGGGGS

SEQ ID NO: 27 - protein, 8 aa, synthetic construct
GFAFSSYD

SEQ ID NO: 28 - protein, 8 aa, synthetic construct
ISGGGRYT

SEQ ID NO: 29 - protein, 11 aa, synthetic construct
ANRYGEAWFAY

SEQ ID NO: 30 - protein, 6 aa, synthetic construct
QDINTY

SEQ ID NO: 31 - skipped

SEQ ID NO: 32 - protein, 9 aa, synthetic construct
LQYDEFPLT

SEQ ID NO: 33 - protein, 8 aa, synthetic construct
GYSFTGYT

SEQ ID NO: 34 - protein, 8 aa, synthetic construct
INPYNNIT

SEQ ID NO: 35 - protein, 8 aa, synthetic construct
ARLDYRSY

SEQ ID NO: 36 - protein, 9 aa, synthetic construct
TGAVTTSNF

SEQ ID NO: 37 - skipped

SEQ ID NO: 38 - protein, 9 aa, synthetic construct
ALWYSNHWV

SEQ ID NO: 39 - DNA, 1344 bp, synthetic construct
  source 1..1344: mol_type = other DNA
gaagtgcagctggtcgagtctgggggagggctggtgcagcccggcgggtcactgcgactgagctgcgcagcttccggattcgcctttagctcctacgacatgtcctgggtgcgacaggcaccaggaaagggactggattgggtcgctactatctcaggaggcgggagatacacctactatcctgacagcgtcaagggccggttcacaatctctagagataacagtaagaacaatctgtatctgcagatgaacagcctgagggctgaggacaccgcactgtactattgtgccaaccgctacggggaagcatggtttgcctattgggggcagggaaccctggtgacagtctctagtgccagcaccaaagggcccagcgtgtttcctctcgccccctcctccaaaagcaccagcggaggaaccgctgctctcggatgtctggtgaaggactacttccctgaacccgtcaccgtgagctggaatagcggcgctctgacaagcggagtccatacattccctgctgtgctgcaaagcagcggactctattccctgtccagcgtcgtcacagtgcccagcagcagcctgggcacccagacctacatctgtaacgtcaaccacaagccctccaacaccaaggtggacaagaaagtggagcccaaatcctgcgacaagacacacacctgtcccccctgtcctgctcccgaagctgctggagcccctagcgtcttcctctttcctcccaaacccaaggacaccctcatgatcagcagaacccctgaagtcacctgtgtcgtcgtggatgtcagccatgaggaccccgaggtgaaattcaactggtatgtcgatggcgtcgaggtgcacaacgccaaaaccaagcccagggaggaacagtacaactccacctacagggtggtgtccgtgctgacagtcctccaccaggactggctgaacggcaaggagtacaagtgcaaggtgtccaacaaggctctccctgcccccattgagaagaccatcagcaaggccaaaggccaacccagggagccccaggtctatacactgcctccctccagggacgaactcaccaagaaccaggtgtccctgacctgcctggtcaagggcttttatcccagcgacatcgccgtcgagtgggagtccaacggacagcccgagaataactacaagaccacccctcctgtcctcgactccgacggctccttcttcctgtacagcaagctgaccgtggacaaaagcaggtggcagcagggaaacgtgttctcctgcagcgtgatgcacgaagccctccacaaccactacacccagaaaagcctgtccctgagccccggcaaa

SEQ ID NO: 40 - protein, 448 aa, synthetic construct
EVQLVESGGGLVQPGGSLRLSCAASGFAFSSYDMSWVRQAPGKGLDWVATISGGGRYTYYPDSVKGRFTISRDNSKNNLYLQMNSLRAEDTALYYCANRYGEAWFAYWGQGTLVTVSSASTKGPSVFPLAPSSKSTSGGTAALGCLVKDYFPEPVTVSWNSGALTSGVHTFPAVLQSSGLYSLSSVVTVPSSSLGTQTYICNVNHKPSNTKVDKKVEPKSCDKTHTCPPCPAPEAAGAPSVFLFPPKPKDTLMISRTPEVTCVVVDVSHEDPEVKFNWYVDGVEVHNAKTKPREEQYNSTYRVVSVLTVLHQDWLNGKEYKCKVSNKALPAPIEKTISKAKGQPREPQVYTLPPSRDELTKNQVSLTCLVKGFYPSDIAVEWESNGQPENNYKTTPPVLDSDGSFFLYSKLTVDKSRWQQGNVFSCSVMHEALHNHYTQKSLSLSPGK

SEQ ID NO: 41 - protein, 115 aa, synthetic construct
QVQLVESGAELVKPGASMKISCKASGYSFTGYTMNWVKQAPGQCLEWIGLINPYNNITNYNQKFMGKATFTVDKSISTAYMELSRLTSDDSGVYFCARLDYRSYWGQGTLVTVSA

SEQ ID NO: 42 - protein, 110 aa, synthetic construct
QAVVTQEPSLTVSPGGTVTLTCGSSTGAVTTSNFANWVQEKPGQAFRSLIGGTNNRASWVPARFSGSLLGGKAALTISGAQPEDEAEYFCALWYSNHWVFGCGTKLTVLR

SEQ ID NO: 43 - protein, 115 aa, synthetic construct
QVQLVESGAEVKKPGASVKVSCKASGYSFTGYTMNWVRQAPGQCLEWIGLINPYNNITNYAQKFQGRVTFTVDTSISTAYMELSRLRSDDTGVYFCARLDYRSYWGQGTLVTVSA

SEQ ID NO: 44 - protein, 110 aa, synthetic construct
QAVVTQEPSLTVSPGGTVTLTCGSSTGAVTTSNFPNWVQQKPGQAPRSLIGGTNNKASWTPARFSGSLLGGKAALTISGAQPEDEAEYYCALWYSNHWVFGCGTKLTVLR

SEQ ID NO: 45 - protein, 5 aa, synthetic construct
GGGGS